European Patent Application EP 4 786 590 A1, published August 5, 2026. Title: Nucleic acid molecule comprising modified polyadenyl sequence. Applicant: HANMI PHARM. CO., LTD. The sequence listing filed with the application follows.

SEQUENCE LISTING (32 sequences)

SEQ ID NO: 1 - DNA, 158 bp, Homo sapiens
  source 1..158: mol_type = genomic DNA
gtgtgtggaggacaccctgaaccccccgctttcaaacaagttttcaaattgtttgaggtcaggatttctcaaactgattcctttctttgcatatgagtatttgaaaataaatattttcccagaatataaataaatcatcacatgattattttaactat

SEQ ID NO: 2 - DNA, 142 bp, synthetic construct
  source 1..142: mol_type = other DNA
aaaaaaaaaaaaaaaaaaaaacaaccagctaagacactgccaaaaaaaaaaaaaaaaaaaaaaaaaaaaaaaaaaaaaaaaaaaaaaaaaaaaaaaaaaaaaaaaaaaaaaaaaaaaaaaaaaaaaaaaaaaaaaaaaaaaa

SEQ ID NO: 3 - DNA, 3103 bp, synthetic construct
  source 1..3103: mol_type = other DNA
aagcttctcgaggtgtgtggaggacaccctgaaccccccgctttcaaacaagttttcaaattgtttgaggtcaggatttctcaaactgattcctttctttgcatatgagtatttgaaaataaatattttcccagaatataaataaatcatcacatgattattttaactatgctagcaaaaaaaaaaaaaaaaaaaaacaaccagctaagacactgccaaaaaaaaaaaaaaaaaaaaaaaaaaaaaaaaaaaaaaaaaaaaaaaaaaaaaaaaaaaaaaaaaaaaaaaaaaaaaaaaaaaaaaaaaaaaaaaaaaaaagaagagcgaattcactggccgtcgttttacagttacccaacttaatcgcctcgcctgatgcggtattttctccttacgcatctgtgcggtatttcacaccgcatatggtgcactctcagtacaatctgctctgatgccgcatagttaagccagccccgacacccgccaacacccgctgacgcgccctgacgggcttgtctgctcccggcatccgcttacagacaagctgtgaccgtctccgggagctgcatgtgtcagaggttttcaccgtcatcaccgaaacgcgcgagacgaaagggcctcgtgatacgcctatttttataggttaatgtcatgataataatggtttcttagacgtcaggtggcacttttcggggaaatgtgcgcggaacccctatttgtttatttttctaaatacattcaaatatgtatccgctcatgagacaataaccctgataaatgcttcaataatattgaaaaagtatgagtattcaacatttccgtgtcgcccttattcccttttttgcggcattttgccttcctgtttttgctcacccagaaacgctggtgaaagtaaaagatgctgaagatcagttgggtgcacgagtgggttacatcgaactggatctcaacagcggtaagatccttgagagttttcgccccgaagaacgttttccatgcagctctggcccgtgtctcaaaatctctgatgttacattgcacaagataaaaatatatcatcatgaacaataaaactgtctgcttacataaacagtaatacaaggggtgttatgagccatattcaacgggaaacgtcgaggccgcgattaaattccaacatggatgctgatttatatgggtataaatgggctcgcgataatgtcgggcaatcaggtgcgacaatctatcgcttgtatgggaagcccgatgcgccagagttgtttctgaaacatggcaaaggtagcgttgccaatgatgttacagatgagatggtcagactaaactggctgacggaatttatgcctcttccgaccatcaagcattttatccgtactcctgatgatgcatggttactcaccactgcgatccccggaaaaacagcattccaggtattagaagaatatcctgattcaggtgaaaatattgttgatgcgctggcagtgttcctgcgccggttgcattcgattcctgtttgtaattgtccttttaacagcgatcgcgtatttcgtctcgctcaggcgcaatcacgaatgaataacggtttggttgatgcgagtgattttgatgacgagcgtaatggctggcctgttgaacaagtctggaaagaaatgcataaacttttgccattctcaccggattcagtcgtcactcatggtgatttctcacttgataaccttatttttgacgaggggaaattaataggttgtattgatgttggacgagtcggaatcgcagaccgataccaggatcttgccatcctatggaactgcctcggtgagttttctccttcattacagaaacggctttttcaaaaatatggtattgataatcctgatatgaataaattgcagtttcatttgatgctcgatgagtttttctaatcagaattggttaattggttgtaacattattcagattgggcttgatttaaaacttcatttttaatttaaaaggatctaggtgaagatcctttttgataatctcatgaccaaaatcccttaacgtgagttttcgttccactgagcgtcagaccccgtagaaaagatcaaaggatcttcttgagatcctttttttctgcgcgtaatctgctgcttgcaaacaaaaaaaccaccgctaccagcggtggtttgtttgccggatcaagagctaccaactctttttccgaaggtaactggcttcagcagagcgcagataccaaatactgttcttctagtgtagccgtagttaggccaccacttcaagaactctgtagcaccgcctacatacctcgctctgctaatcctgttaccagtggctgctgccagtggcgataagtcgtgtcttaccgggttggactcaagacgatagttaccggataaggcgcagcggtcgggctgaacggggggttcgtgcacacagcccagcttggagcgaacgacctacaccgaactgagatacctacagcgtgagctatgagaaagcgccacgcttcccgaagggagaaaggcggacaggtatccggtaagcggcagggtcggaacaggagagcgcacgagggagcttccagggggaaacgcctggtatctttatagtcctgtcgggtttcgccacctctgacttgagcgtcgatttttgtgatgctcgtcaggggggcggagcctatggaaaaacgccagcaacgcggcctttttacggttcctggccttttgctggccttttgcgagccttttgctcacatgttctttcctgcgttatcccctgattctgtggataaccgtattaccgcctttgagtgagctgataccgctcgccgcagccgaacgaccgagcgcagcgagtcagtgagcgaggaagcggcccaatacgcaaaccgcctctccccgcgcgttggccgattcattaatgcagctggcacgacaggtttcccgactggaaagcgggcagtgagcgcaacgcaattaatgtgagttagctcactcattaggcaccccaggctttacactttatgcttccggctcgtatgttgtgtggaattgtgagcggataacaatttcacacaggaaacagctatgaccatgattacgcc

SEQ ID NO: 4 - DNA, 3079 bp, synthetic construct
  source 1..3079: mol_type = other DNA
gtgtgtggaggacaccctgaaccccccgctttcaaacaagttttcaaattgtttgaggtcaggatttctcaaactgattcctttctttgcatatgagtatttgaaaataaatattttcccagaatataaataaatcatcacatgattattttaactataaaaaaaaaaaaaaaaaaaaacaaccagctaagacactgccaaaaaaaaaaaaaaaaaaaaaaaaaaaaaaaaaaaaaaaaaaaaaaaaaaaaaaaaaaaaaaaaaaaaaaaaaaaaaaaaaaaaaaaaaaaaaaaaaaaaagaagagcactggccgtcgttttacagttacccaacttaatcgcctcgcctgatgcggtattttctccttacgcatctgtgcggtatttcacaccgcatatggtgcactctcagtacaatctgctctgatgccgcatagttaagccagccccgacacccgccaacacccgctgacgcgccctgacgggcttgtctgctcccggcatccgcttacagacaagctgtgaccgtctccgggagctgcatgtgtcagaggttttcaccgtcatcaccgaaacgcgcgagacgaaagggcctcgtgatacgcctatttttataggttaatgtcatgataataatggtttcttagacgtcaggtggcacttttcggggaaatgtgcgcggaacccctatttgtttatttttctaaatacattcaaatatgtatccgctcatgagacaataaccctgataaatgcttcaataatattgaaaaagtatgagtattcaacatttccgtgtcgcccttattcccttttttgcggcattttgccttcctgtttttgctcacccagaaacgctggtgaaagtaaaagatgctgaagatcagttgggtgcacgagtgggttacatcgaactggatctcaacagcggtaagatccttgagagttttcgccccgaagaacgttttccatgcagctctggcccgtgtctcaaaatctctgatgttacattgcacaagataaaaatatatcatcatgaacaataaaactgtctgcttacataaacagtaatacaaggggtgttatgagccatattcaacgggaaacgtcgaggccgcgattaaattccaacatggatgctgatttatatgggtataaatgggctcgcgataatgtcgggcaatcaggtgcgacaatctatcgcttgtatgggaagcccgatgcgccagagttgtttctgaaacatggcaaaggtagcgttgccaatgatgttacagatgagatggtcagactaaactggctgacggaatttatgcctcttccgaccatcaagcattttatccgtactcctgatgatgcatggttactcaccactgcgatccccggaaaaacagcattccaggtattagaagaatatcctgattcaggtgaaaatattgttgatgcgctggcagtgttcctgcgccggttgcattcgattcctgtttgtaattgtccttttaacagcgatcgcgtatttcgtctcgctcaggcgcaatcacgaatgaataacggtttggttgatgcgagtgattttgatgacgagcgtaatggctggcctgttgaacaagtctggaaagaaatgcataaacttttgccattctcaccggattcagtcgtcactcatggtgatttctcacttgataaccttatttttgacgaggggaaattaataggttgtattgatgttggacgagtcggaatcgcagaccgataccaggatcttgccatcctatggaactgcctcggtgagttttctccttcattacagaaacggctttttcaaaaatatggtattgataatcctgatatgaataaattgcagtttcatttgatgctcgatgagtttttctaatcagaattggttaattggttgtaacattattcagattgggcttgatttaaaacttcatttttaatttaaaaggatctaggtgaagatcctttttgataatctcatgaccaaaatcccttaacgtgagttttcgttccactgagcgtcagaccccgtagaaaagatcaaaggatcttcttgagatcctttttttctgcgcgtaatctgctgcttgcaaacaaaaaaaccaccgctaccagcggtggtttgtttgccggatcaagagctaccaactctttttccgaaggtaactggcttcagcagagcgcagataccaaatactgttcttctagtgtagccgtagttaggccaccacttcaagaactctgtagcaccgcctacatacctcgctctgctaatcctgttaccagtggctgctgccagtggcgataagtcgtgtcttaccgggttggactcaagacgatagttaccggataaggcgcagcggtcgggctgaacggggggttcgtgcacacagcccagcttggagcgaacgacctacaccgaactgagatacctacagcgtgagctatgagaaagcgccacgcttcccgaagggagaaaggcggacaggtatccggtaagcggcagggtcggaacaggagagcgcacgagggagcttccagggggaaacgcctggtatctttatagtcctgtcgggtttcgccacctctgacttgagcgtcgatttttgtgatgctcgtcaggggggcggagcctatggaaaaacgccagcaacgcggcctttttacggttcctggccttttgctggccttttgcgagccttttgctcacatgttctttcctgcgttatcccctgattctgtggataaccgtattaccgcctttgagtgagctgataccgctcgccgcagccgaacgaccgagcgcagcgagtcagtgagcgaggaagcggcccaatacgcaaaccgcctctccccgcgcgttggccgattcattaatgcagctggcacgacaggtttcccgactggaaagcgggcagtgagcgcaacgcaattaatgtgagttagctcactcattaggcaccccaggctttacactttatgcttccggctcgtatgttgtgtggaattgtgagcggataacaatttcacacaggaaacagctatgaccatgattacgcc

SEQ ID NO: 5 - DNA, 17 bp, synthetic construct
  source 1..17: mol_type = other DNA
taatacgactcactata

SEQ ID NO: 6 - DNA, 61 bp, synthetic construct
  source 1..61: mol_type = other DNA
agtgctccccatccaactaaactgtccctctgtccgaactaaactgcactgtcccagcacc

SEQ ID NO: 7 - DNA, 1179 bp, Homo sapiens
  source 1..1179: mol_type = genomic DNA
atggaagaacctcagtccgatccgagcgtcgagcctcccctgtcacaggaaactttcagtgacctgtggaaactgctgcccgagaataatgtactttcgcctctgcctagccaagcaatggatgatctgatgctgtctccagatgacatcgaacagtggtttacagaggatccagggcccgatgaggcaccacgaatgccagaggcggccccacctgttgcacccgcacctgcggctccaacacccgcagcccccgcccccgctccaagctggcctctcagtagttccgtgccatcacagaagacctatcaaggcagctacggatttcgcctcggatttctccattcaggcactgccaagtccgtgacttgtacgtacagccccgctctgaacaaaatgttctgtcagttggcgaagacatgtcctgtccagctttgggtagattctacccccccgccggggacacgggtgcgagccatggccatttataaacagtctcagcacatgaccgaggtcgtgcgcaggtgtcctcaccatgaacgatgctccgactccgacggcctggcccccccacagcacctgattcgcgtggaaggcaatcttcgtgtggagtacctcgatgatcggaacaccttcagacatagcgtggttgtgccttatgagccacccgaagttggaagcgactgtaccaccatccattacaactatatgtgcaacagtagctgcatgggtggcatgaatcggcggcctatcttgacaataatcactttagaggactcttccggaaacctgcttggcagaaattcattcgaggtccgtgtctgcgcctgcccgggcagggaccgcagaaccgaagaggagaatttacggaaaaagggggaaccccaccacgaactgccaccgggcagtaccaaaagggctctccctaataacacatcttcatcgccccagccaaagaagaaacccctcgacggagagtactttactctacaaattagggggagagaaagatttgagatgttccgcgaattgaacgaggccctggagttgaaagacgctcaagccggaaaggaaccaggtgggtctagggcccactcaagccatctgaagagtaagaaaggccagtccacttccaggcacaaaaagttaatgttcaagacggagggtcctgactctgac

SEQ ID NO: 8 - RNA, 61 nt, synthetic construct
  source 1..61: mol_type = other RNA
agtgctccccatccaactaaactgtccctctgtccgaactaaactgcactgtcccagcacc

SEQ ID NO: 9 - RNA, 1185 nt, Homo sapiens
  source 1..1185: mol_type = mRNA
atggaagaacctcagtccgatccgagcgtcgagcctcccctgtcacaggaaactttcagtgacctgtggaaactgctgcccgagaataatgtactttcgcctctgcctagccaagcaatggatgatctgatgctgtctccagatgacatcgaacagtggtttacagaggatccagggcccgatgaggcaccacgaatgccagaggcggccccacctgttgcacccgcacctgcggctccaacacccgcagcccccgcccccgctccaagctggcctctcagtagttccgtgccatcacagaagacctatcaaggcagctacggatttcgcctcggatttctccattcaggcactgccaagtccgtgacttgtacgtacagccccgctctgaacaaaatgttctgtcagttggcgaagacatgtcctgtccagctttgggtagattctacccccccgccggggacacgggtgcgagccatggccatttataaacagtctcagcacatgaccgaggtcgtgcgcaggtgtcctcaccatgaacgatgctccgactccgacggcctggcccccccacagcacctgattcgcgtggaaggcaatcttcgtgtggagtacctcgatgatcggaacaccttcagacatagcgtggttgtgccttatgagccacccgaagttggaagcgactgtaccaccatccattacaactatatgtgcaacagtagctgcatgggtggcatgaatcggcggcctatcttgacaataatcactttagaggactcttccggaaacctgcttggcagaaattcattcgaggtccgtgtctgcgcctgcccgggcagggaccgcagaaccgaagaggagaatttacggaaaaagggggaaccccaccacgaactgccaccgggcagtaccaaaagggctctccctaataacacatcttcatcgccccagccaaagaagaaacccctcgacggagagtactttactctacaaattagggggagagaaagatttgagatgttccgcgaattgaacgaggccctggagttgaaagacgctcaagccggaaaggaaccaggtgggtctagggcccactcaagccatctgaagagtaagaaaggccagtccacttccaggcacaaaaagttaatgttcaagacggagggtcctgactctgacctcgag

SEQ ID NO: 10 - RNA, 164 nt, synthetic construct
  source 1..164: mol_type = other RNA
gtgtgtggaggacaccctgaaccccccgctttcaaacaagttttcaaattgtttgaggtcaggatttctcaaactgattcctttctttgcatatgagtatttgaaaataaatattttcccagaatataaataaatcatcacatgattattttaactatgctagc

SEQ ID NO: 11 - RNA, 155 nt, synthetic construct
  source 1..155: mol_type = other RNA
aaaaaaaaaaaaaaaaaaaaacaaccagctaagacactgccaaaaaaaaaaaaaaaaaaaaaaaaaaaaaaaaaaaaaaaaaaaaaaaaaaaaaaaaaaaaaaaaaaaaaaaaaaaaaaaaaaaaaaaaaaaaaaaaaaaaaagaagagcgaatt

SEQ ID NO: 12 - RNA, 1179 nt, Homo sapiens
  source 1..1179: mol_type = mRNA
atggaagaacctcagtccgatccgagcgtcgagcctcccctgtcacaggaaactttcagtgacctgtggaaactgctgcccgagaataatgtactttcgcctctgcctagccaagcaatggatgatctgatgctgtctccagatgacatcgaacagtggtttacagaggatccagggcccgatgaggcaccacgaatgccagaggcggccccacctgttgcacccgcacctgcggctccaacacccgcagcccccgcccccgctccaagctggcctctcagtagttccgtgccatcacagaagacctatcaaggcagctacggatttcgcctcggatttctccattcaggcactgccaagtccgtgacttgtacgtacagccccgctctgaacaaaatgttctgtcagttggcgaagacatgtcctgtccagctttgggtagattctacccccccgccggggacacgggtgcgagccatggccatttataaacagtctcagcacatgaccgaggtcgtgcgcaggtgtcctcaccatgaacgatgctccgactccgacggcctggcccccccacagcacctgattcgcgtggaaggcaatcttcgtgtggagtacctcgatgatcggaacaccttcagacatagcgtggttgtgccttatgagccacccgaagttggaagcgactgtaccaccatccattacaactatatgtgcaacagtagctgcatgggtggcatgaatcggcggcctatcttgacaataatcactttagaggactcttccggaaacctgcttggcagaaattcattcgaggtccgtgtctgcgcctgcccgggcagggaccgcagaaccgaagaggagaatttacggaaaaagggggaaccccaccacgaactgccaccgggcagtaccaaaagggctctccctaataacacatcttcatcgccccagccaaagaagaaacccctcgacggagagtactttactctacaaattagggggagagaaagatttgagatgttccgcgaattgaacgaggccctggagttgaaagacgctcaagccggaaaggaaccaggtgggtctagggcccactcaagccatctgaagagtaagaaaggccagtccacttccaggcacaaaaagttaatgttcaagacggagggtcctgactctgac

SEQ ID NO: 13 - RNA, 158 nt, Homo sapiens
  source 1..158: mol_type = mRNA
gtgtgtggaggacaccctgaaccccccgctttcaaacaagttttcaaattgtttgaggtcaggatttctcaaactgattcctttctttgcatatgagtatttgaaaataaatattttcccagaatataaataaatcatcacatgattattttaactat

SEQ ID NO: 14 - RNA, 142 nt, synthetic construct
  source 1..142: mol_type = other RNA
aaaaaaaaaaaaaaaaaaaaacaaccagctaagacactgccaaaaaaaaaaaaaaaaaaaaaaaaaaaaaaaaaaaaaaaaaaaaaaaaaaaaaaaaaaaaaaaaaaaaaaaaaaaaaaaaaaaaaaaaaaaaaaaaaaaaa

SEQ ID NO: 15 - protein, 393 aa, Homo sapiens [sequence omitted]

SEQ ID NO: 16 - DNA, 57 bp, Homo sapiens
  source 1..57: mol_type = genomic DNA
atgacaaggttgacggtcctggcattgcttgccgggcttttggcgagttctcgggcg

SEQ ID NO: 17 - DNA, 444 bp, Homo sapiens
  source 1..444: mol_type = genomic DNA
agcagttcacctgcaaaggaccccccaatccagcgactgagaggcgcagtcacccggtgtgaagatggacagctttttatatcatcttacaagaatgagtatcagactatggaggttcaaaataactccgtggttataaagtgcgacgggctttacatcatctatctgaaggggtcctttttccaggaggtcaagatagatttgcacttcagggaagaccataaccccatttctattcctatgcttaatgacggacgacggatcgtatttactgttgtggcttctctcgcttttaaggacaaggtctaccttaccgtgaatgccccagacacactttgcgagcacctccagatcaacgacggagagcttatcgttgttcaacttacaccaggttattgcgctccagaggggagctatcactccaccgtcaaccaggtacccctt

SEQ ID NO: 18 - DNA, 30 bp, synthetic construct
  source 1..30: mol_type = other DNA
ggtggaggcggttcaggcggaggtggctct

SEQ ID NO: 19 - DNA, 60 bp, synthetic construct
  source 1..60: mol_type = other DNA
agcgagagaaaggcccttcagacagaaatggcacgcataaaaaaatggcttacattcagt

SEQ ID NO: 20 - DNA, 441 bp, Homo sapiens
  source 1..441: mol_type = genomic DNA
caggactccgaagcagcaataaaccgacaaataaatctggagttgtacgcatcctacgtttacctgtccatgtcttactacttcgatagagacgatgtcgccctcaaaaacttcgccaagtatttcctgcatcagtcccatgaagagagagagcacgcagagaaactgatgaaacttcagaaccaacgggggggcaggatctttctgcaagacattaagaagcctgattgcgatgactgggaatctggacttaatgccatggagtgtgccctgcacctcgaaaaaaatgtgaaccagagcctgttggaattgcataagctggcaaccgataagaacgatccacatctttgcgatttcatcgaaacccactatctcaatgaacaagtgaaggcaattaaggagctgggcgatcatgtaacaaatttgcgaaaaatgggtgcc

SEQ ID NO: 21 - DNA, 312 bp, Homo sapiens
  source 1..312: mol_type = genomic DNA
tctggctctcagacttgtgaagatacccttaagacttgcagtgtcatagcctgtgggcgagacgggcgcgatggacccaagggcgaaaaaggagaaccagggcaagggctcagaggactgcaaggtccacctggtaaattggggccacctggaagcgtggggtccccaggaagtccaggcccaaaaggtcagaaaggggaccacggcgataatcgagccattgaggaaaaactcgcaaatatggaggccgaaattaggattctgaagagtaagttgcagctgaccaacaagctccatgcttttagcatgggc

SEQ ID NO: 22 - RNA, 57 nt, Homo sapiens
  source 1..57: mol_type = mRNA
atgacaaggttgacggtcctggcattgcttgccgggcttttggcgagttctcgggcg

SEQ ID NO: 23 - RNA, 444 nt, Homo sapiens
  source 1..444: mol_type = mRNA
agcagttcacctgcaaaggaccccccaatccagcgactgagaggcgcagtcacccggtgtgaagatggacagctttttatatcatcttacaagaatgagtatcagactatggaggttcaaaataactccgtggttataaagtgcgacgggctttacatcatctatctgaaggggtcctttttccaggaggtcaagatagatttgcacttcagggaagaccataaccccatttctattcctatgcttaatgacggacgacggatcgtatttactgttgtggcttctctcgcttttaaggacaaggtctaccttaccgtgaatgccccagacacactttgcgagcacctccagatcaacgacggagagcttatcgttgttcaacttacaccaggttattgcgctccagaggggagctatcactccaccgtcaaccaggtacccctt

SEQ ID NO: 24 - RNA, 30 nt, synthetic construct
  source 1..30: mol_type = other RNA
ggtggaggcggttcaggcggaggtggctct

SEQ ID NO: 25 - RNA, 60 nt, synthetic construct
  source 1..60: mol_type = other RNA
agcgagagaaaggcccttcagacagaaatggcacgcataaaaaaatggcttacattcagt

SEQ ID NO: 26 - RNA, 441 nt, Homo sapiens
  source 1..441: mol_type = mRNA
caggactccgaagcagcaataaaccgacaaataaatctggagttgtacgcatcctacgtttacctgtccatgtcttactacttcgatagagacgatgtcgccctcaaaaacttcgccaagtatttcctgcatcagtcccatgaagagagagagcacgcagagaaactgatgaaacttcagaaccaacgggggggcaggatctttctgcaagacattaagaagcctgattgcgatgactgggaatctggacttaatgccatggagtgtgccctgcacctcgaaaaaaatgtgaaccagagcctgttggaattgcataagctggcaaccgataagaacgatccacatctttgcgatttcatcgaaacccactatctcaatgaacaagtgaaggcaattaaggagctgggcgatcatgtaacaaatttgcgaaaaatgggtgcc

SEQ ID NO: 27 - RNA, 170 nt, synthetic construct
  source 1..170: mol_type = other RNA
ctcgaggtgtgtggaggacaccctgaaccccccgctttcaaacaagttttcaaattgtttgaggtcaggatttctcaaactgattcctttctttgcatatgagtatttgaaaataaatattttcccagaatataaataaatcatcacatgattattttaactatgctagc

SEQ ID NO: 28 - RNA, 312 nt, Homo sapiens
  source 1..312: mol_type = other RNA
tctggctctcagacttgtgaagatacccttaagacttgcagtgtcatagcctgtgggcgagacgggcgcgatggacccaagggcgaaaaaggagaaccagggcaagggctcagaggactgcaaggtccacctggtaaattggggccacctggaagcgtggggtccccaggaagtccaggcccaaaaggtcagaaaggggaccacggcgataatcgagccattgaggaaaaactcgcaaatatggaggccgaaattaggattctgaagagtaagttgcagctgaccaacaagctccatgcttttagcatgggc

SEQ ID NO: 29 - protein, 349 aa, synthetic construct
MTRLTVLALLAGLLASSRASSSPAKDPPIQRLRGAVTRCEDGQLFISSYKNEYQTMEVQNNSVVIKCDGLYIIYLKGSFFQEVKIDLHFREDHNPISIPMLNDGRRIVFTVVASLAFKDKVYLTVNAPDTLCEHLQINDGELIVVQLTPGYCAPEGSYHSTVNQVPLGGGGSGGGGSSERKALQTEMARIKKWLTFSGGGGSQDSEAAINRQINLELYASYVYLSMSYYFDRDDVALKNFAKYFLHQSHEEREHAEKLMKLQNQRGGRIFLQDIKKPDCDDWESGLNAMECALHLEKNVNQSLLELHKLATDKNDPHLCDFIETHYLNEQVKAIKELGDHVTNLRKMGA

SEQ ID NO: 30 - protein, 281 aa, synthetic construct
MTRLTVLALLAGLLASSRASGSQTCEDTLKTCSVIACGRDGRDGPKGEKGEPGQGLRGLQGPPGKLGPPGSVGSPGSPGPKGQKGDHGDNRAIEEKLANMEAEIRILKSKLQLTNKLHAFSMGGGGGSGGGGSSSSPAKDPPIQRLRGAVTRCEDGQLFISSYKNEYQTMEVQNNSVVIKCDGLYIIYLKGSFFQEVKIDLHFREDHNPISIPMLNDGRRIVFTVVASLAFKDKVYLTVNAPDTLCEHLQINDGELIVVQLTPGYCAPEGSYHSTVNQVPL

SEQ ID NO: 31 - DNA, 15 bp, synthetic construct
  source 1..15: mol_type = other DNA
ggtggaggcggttca

SEQ ID NO: 32 - RNA, 15 nt, synthetic construct
  source 1..15: mol_type = other RNA
ggtggaggcggttca